European Patent Application EP 4 186 918 A1, published May 31, 2023. Title: Inhibitory Peptides for the Diagnostic and/or Treatment of Tauopathies. Applicant: Université de Rennes Cyrille, GARNIER. The sequence listing filed with the application follows.

SEQUENCE LISTING (51 sequences)

SEQ ID NO: 1 - protein, 6 aa, Homo sapiens
VQIINK

SEQ ID NO: 2 - protein, 6 aa, Homo sapiens
VQIVYK

SEQ ID NO: 3 - protein, 5 aa, Homo sapiens
HKLTF

SEQ ID NO: 4 - protein, 6 aa, Homo sapiens
QVEVKS

SEQ ID NO: 5 - protein, 6 aa, Artificial Sequence
  Peptide 3p
VKYQVI

SEQ ID NO: 6 - protein, 6 aa, Artificial Sequence
  Peptide 4p
VQKIYV

SEQ ID NO: 7 - protein, 6 aa, Artificial Sequence
  Peptide 5p
IKQVYV

SEQ ID NO: 8 - protein, 6 aa, Artificial Sequence
  Peptide 6p
VVQKYI

SEQ ID NO: 9 - protein, 6 aa, Artificial Sequence
  Peptide 8p
QKYIVV

SEQ ID NO: 10 - protein, 6 aa, Artificial Sequence
  Peptide 9p
IYVQKV

SEQ ID NO: 11 - protein, 6 aa, Artificial Sequence
  Peptide 13p
YIVVQK

SEQ ID NO: 12 - protein, 6 aa, Artificial Sequence
  Peptide 14p
KVQYVI

SEQ ID NO: 13 - protein, 6 aa, Artificial Sequence
  Peptide 23 p
QVIKYV

SEQ ID NO: 14 - protein, 6 aa, Artificial Sequence
  Peptide 1tp
VKIVYQ

SEQ ID NO: 15 - protein, 6 aa, Artificial Sequence
  Peptide 4tp
VKIQYV

SEQ ID NO: 16 - protein, 6 aa, Artificial Sequence
  Peptide 6tp
YQIVVK

SEQ ID NO: 17 - protein, 6 aa, Artificial Sequence
  Peptide 3pinv
IVQYKV

SEQ ID NO: 18 - protein, 6 aa, Artificial Sequence
  Peptide 4pinv
VYIKQV

SEQ ID NO: 19 - protein, 6 aa, Artificial Sequence
  Peptide 5pinv
VYVQKI

SEQ ID NO: 20 - protein, 6 aa, Artificial Sequence
  Peptide 6pinv
IYKQVV

SEQ ID NO: 21 - protein, 6 aa, Artificial Sequence
  Peptide 8pinv
VVIYKQ

SEQ ID NO: 22 - protein, 6 aa, Artificial Sequence
  Peptide 9pinv
VKQVYI

SEQ ID NO: 23 - protein, 6 aa, Artificial Sequence
  Peptide 13pinv
KQVVIY

SEQ ID NO: 24 - protein, 6 aa, Artificial Sequence
  Peptide 14pinv
IVYQVK

SEQ ID NO: 25 - protein, 6 aa, Artificial Sequence
  Peptide 23pinv
VYKIVQ

SEQ ID NO: 26 - protein, 6 aa, Artificial Sequence
  Peptide 1tpinv
QYVIKV

SEQ ID NO: 27 - protein, 6 aa, Artificial Sequence
  Peptide 4tpinv
VYQIKV

SEQ ID NO: 28 - protein, 6 aa, Artificial Sequence
  Peptide 6tpinv
KVVIQY

SEQ ID NO: 29 - protein, 6 aa, Artificial Sequence
  Peptide 1p
VQIVYK

SEQ ID NO: 30 - protein, 6 aa, Artificial Sequence
  Peptide 2p
KYIQVV

SEQ ID NO: 31 - protein, 6 aa, Artificial Sequence
  Peptide 7p
VKVIYQ

SEQ ID NO: 32 - protein, 6 aa, Artificial Sequence
  Peptide 9p
IYVQKV

SEQ ID NO: 33 - protein, 6 aa, Artificial Sequence
  Peptide 10p
KVQIVY

SEQ ID NO: 34 - protein, 6 aa, Artificial Sequence
  Peptide 11p
VKVYIQ

SEQ ID NO: 35 - protein, 6 aa, Artificial Sequence
  Peptide 12p
VQVIYK

SEQ ID NO: 36 - protein, 6 aa, Artificial Sequence
  Peptide 15p
KYVIQV

SEQ ID NO: 37 - protein, 6 aa, Artificial Sequence
  Peptide 16p
YQVKIV

SEQ ID NO: 38 - protein, 6 aa, Artificial Sequence
  Peptide 17p
YQVIVK

SEQ ID NO: 39 - protein, 6 aa, Artificial Sequence
  Peptide 18p
QKVVYI

SEQ ID NO: 40 - protein, 6 aa, Artificial Sequence
  Peptide 19p
QKVYIV

SEQ ID NO: 41 - protein, 6 aa, Artificial Sequence
  Peptide 20p
KQIVYV

SEQ ID NO: 42 - protein, 6 aa, Artificial Sequence
  Peptide 21p
VQVKYI

SEQ ID NO: 43 - protein, 6 aa, Artificial Sequence
  Peptide 22p
VQVYKI

SEQ ID NO: 44 - protein, 6 aa, Artificial Sequence
  Peptide 0tp
VQIKYV

SEQ ID NO: 45 - protein, 6 aa, Artificial Sequence
  Peptide 2tp
VVIQYK

SEQ ID NO: 46 - protein, 6 aa, Artificial Sequence
  Peptide 3tp
VVIKYQ

SEQ ID NO: 47 - protein, 6 aa, Artificial Sequence
  Peptide 5tp
VQYVIK

SEQ ID NO: 48 - protein, 6 aa, Artificial Sequence
  Peptide 7tp
IQVVYK

SEQ ID NO: 49 - protein, 6 aa, Artificial Sequence
  Peptide 8tp
IQYVVK

SEQ ID NO: 50 - protein, 6 aa, Artificial Sequence
  Peptide 9tp
YQVVIK

SEQ ID NO: 51 - protein, 11 aa, Artificial Sequence
  Spacer peptide
GPNSKQSQDEG